European Patent Specification EP 3 442 542 B1, published January 29, 2025. Title: NANOPARTICLES, CONTROLLED-RELEASE DOSAGE FORMS, AND METHODS FOR DELIVERING AN IMMUNOTHERAPEUTIC AGENT. Applicant: North Carolina State University. The sequence listing filed with the application follows.

SEQUENCE LISTING (3 sequences)

SEQ ID NO: 1 - DNA, 72 bp, Artificial Sequence
  synthetic construct
gcgcgtcgtcgttcgaacgacgttgcgcgtcgtcgttcgaacgacgttgcgcgtcgtcgttcgaacgacgtt

SEQ ID NO: 2 - DNA, 72 bp, Artificial Sequence
  synthetic construct
atatgtcgtcgttcgaacgacgttatataacgtcgttcgaacgacgttatatgtcgtcgttcgaacgacgtt

SEQ ID NO: 3 - DNA, 72 bp, Artificial Sequence
  synthetic construct
gcgcgtattatttcgaaataatttgcgcgtattatttataaataatttgcgcgtattatttataaataattt